European Patent Specification EP 4 081 655 B1, published March 18, 2026. Title: DISEASE DETECTION IN LIQUID BIOPSIES. Applicant: VIB VZW KATHOLIEKE UNIVERSITEIT LEUVEN, K.U.LEUVEN R&D. The sequence listing filed with the application follows.

SEQUENCE LISTING (2 sequences)

SEQ ID NO: 1 - DNA, 250 bp, Homo sapiens
aggctgcgccacttcctttggggctcgctcgcgcttcctgggagcctttgatgtgggttcttggtagatcctgcccgcggggcctggatgcgggcggagcctccgggcagggcggggcctcagcctgggtccgcactggggaggcggccacccggtagcttgggcgggttccgcccacctcccgcctgtatttacagcccccttccaacatccccgactccctgagggcgcccctcattctgctcggcct

SEQ ID NO: 2 - DNA, 240 bp, Homo sapiens
cgccacttcctttggggctcgctcgcgcttcctgggagcctttgatgtgggttcttggtagatcctgcccgcggggcctggatgcgggcggagcctccgggcagggcggggcctcagcctgggtccgcactggggaggcggccacccggtagcttgggcgggttccgcccacctcccgcctgtatttacagcccccttccaacatccccgactccctgagggcgcccctcattctgctcg